European Patent Application EP 4 180 539 A1, published May 17, 2023. Title: SINGLE END DUPLEX DNA SEQUENCING. Applicant: QIAGEN LIFE SCIENCES, LLC. Application EP EP 17 742 610.3, filed July 11, 2017. The sequence listing filed with the application follows.

SEQUENCE LISTING (12 sequences)

SEQ ID NO: 1 - DNA, 44 bp, synthetic construct
  source 1..44: mol_type = other DNA
  misc_feature 1..44: note = Synthetic complementary double-stranded adaptersequence
  misc_feature 1..44: note = n = A,T,C or G
acactctttccctacacgctcttccgatcnnnnnnnnnngtcat

SEQ ID NO: 2 - DNA, 46 bp, synthetic construct
  source 1..46: mol_type = other DNA
  misc_feature 1..46: note = Synthetic complementary double-stranded adaptersequence
  misc_feature 1..46: note = n = A,T,C or G
tgacnnnnnnnnnngatcggaagagctgagtgtagggaaagagtgt

SEQ ID NO: 3 - DNA, 91 bp, synthetic construct
  source 1..91: mol_type = other DNA
  misc_feature 1..91: note = Synthetic complementary double-stranded adaptersequence
  misc_feature 1..91: note = n = A,T,C or G
aatgatacggcgaccaccgagatctacactctttccctacacgacgctcttccgatctnnnnnnnnnnttcttagcgattattggagtcct

SEQ ID NO: 4 - DNA, 90 bp, synthetic construct
  source 1..90: mol_type = other DNA
  misc_feature 1..90: note = Synthetic complementary double-stranded adaptersequence
  misc_feature 1..90: note = n = A,T,C or G
ggactccaatggtcgctaagaannnnnnnnnnagatcggaagagcgtcgtgtagggaaagagtgtagatctcggtggtcgccgtatcatt

SEQ ID NO: 5 - DNA, 93 bp, synthetic construct
  source 1..93: mol_type = other DNA
  misc_feature 1..93: note = Primer sequence
  misc_feature 1..93: note = n = A,T,C or G
aatgatacggcgaccaccgagatctacactctttccctacacgacgctcttccgatctnnnnnnnnnnnnttctgagcgattataggagtcct

SEQ ID NO: 6 - DNA, 22 bp, synthetic construct
  source 1..22: mol_type = other DNA
  misc_feature 1..22: note = Primer sequence
  modified_base 1: mod_base = OTHER; note = phosphorus
ggactcctatggtcgctcagaa

SEQ ID NO: 7 - DNA, 21 bp, synthetic construct
  source 1..21: mol_type = other DNA
  misc_feature 1..21: note = Primer sequence
aatgtacagtattgcgttttg

SEQ ID NO: 8 - DNA, 20 bp, synthetic construct
  source 1..20: mol_type = other DNA
  misc_feature 1..20: note = Illumina F primer sequence
aatgatacggcgaccaccga

SEQ ID NO: 9 - DNA, 58 bp, synthetic construct
  source 1..58: mol_type = other DNA
  misc_feature 1..58: note = Universal primer (IL2)
aatgatacggcgaccaccgagatctacactctttccctacacgacgctcttccgatct

SEQ ID NO: 10 - DNA, 79 bp, synthetic construct
  source 1..79: mol_type = other DNA
  misc_feature 1..79: note = IL1 ID(#)-RS2 primer
caagcagaagacggcatacgagatgtgactggagttcagacgtgtgctcttccgatctaatgtacagtattgcgttttg

SEQ ID NO: 11 - DNA, 29 bp, synthetic construct
  source 1..29: mol_type = other DNA
  misc_feature 1..29: note = Primer sequence
acactctttccctacacgctcttccgatc

SEQ ID NO: 12 - DNA, 22 bp, synthetic construct
  misc_feature 1..22: note = Primer sequence
  source 1..22: mol_type = other DNA
ggactccaatggtcgctaagaa